European Patent Specification EP 4 032 552 B1, published October 4, 2023. Title: Method and Composition for Enhanced Anti-Tumor Effector Functioning of T Cells. Applicant: Jensen, Michael. The sequence listing filed with the application follows.

SEQUENCE LISTING (53 sequences)

SEQ ID NO: 1 - protein, 132 aa, Homo sapiens
MALLLTTVIALTCLGGFASPGPVPPSTALRYLIEELVNITQNQKAPLCNGSMVWSINLTAGMYCAALESLINVSGCSAIEKTQRMLSGFCPHKVSAGQFSSLHVRDTKIEVAQFVKDLLLHLKKLFREGRFN

SEQ ID NO: 2 - DNA, 416 bp, Homo sapiens
tatgaattcatggcgcttttgttgaccacggtcattgctctcacttgccttggcggctttgcctccccaggccctgtgcctccctctacagccctcaggtacctcattgaggagctggtcaacatcacccagaaccagaaggctccgctctgcaatggcagcatggtatggagcatcaacctgacagctggcatgtactgtgcagccctggaatccctgatcaacgtgtcaggctgcagtgccatcgagaagacccagaggatgctgagcggattctgcccgcacaaggtctcagctgggcagttttccagcttgcatgtccgagacaccaaaatcgaggtggcccagtttgtaaaggacctgctcttacatttaaagaaactttttcgcgagggacggttcaactgaggatccga

SEQ ID NO: 3 - DNA, 416 bp, Homo sapiens
atacttaagtaccgcgaaaacaactggtgccagtaacgagagtgaacggaaccgccgaaacggaggggtccgggacacggagggagatgtcgggagtccatggagtaactcctcgaccagttgtagtgggtcttggtcttccgaggcgagacgttaccgtcgtaccatacctcgtagttggactgtcgaccgtacatgacacgtcgggaccttagggactagttgcacagtccgacgtcacggtagctcttctgggtctcctacgactcgcctaagacgggcgtgttccagagtcgacccgtcaaaaggtcgaacgtacaggctctgtggttttagctccaccgggtcaaacatttcctggacgagaatgtaaatttctttgaaaaagcgctccctgccaagttgactcctaggct

SEQ ID NO: 4 - protein, 497 aa, Homo sapiens
MLLLVTSLLLCELPHPAFLLIPGPVPPSTALRYLIEELVNITQNQKAPLCNGSMVWSINLTAGMYCAALESLINVSGCSAIEKTQRMLSGFCPHKVSAGQFSSLHVRDTKIEVAQFVKDLLLHLKKLFREGRFNESKYGPPCPPCPAPEFLGGPSVFLFPPKPKDTLMISRTPEVTCVVVDVSQEDPEVQFNWYVDGVEVHNAKTKPREEQFNSTYRVVSVLTVLHQDWLNGKEYKCKVSNKGLPSSIEKTISKAKGQPREPQVYTLPPSQEEMTKNQVSLTCLVKGFYPSDIAVEWESNGQPENNYKTTPPVLDSDGSFFLYSRLTVDKSRWQEGNVFSCSVMHEALHNHYTQKSLSLSLGKMALIVLGGVAGLLLFIGLGIFFRVKFSRSADAPAYQQGQNQLYNELNLGRREEYDVLDKRRGRDPEMGGKPRRKNPQEGLYNELQKDKMAEAYSEIGMKGERRRGKGHDGLYQGLSTATKDTYDALHMQALPPR

SEQ ID NO: 5 - DNA, 1522 bp, Homo sapiens
atctctagagccgccaccatgcttctcctggtgacaagccttctgctctgtgagttaccacacccagcattcctcctgatcccaggccctgtgcctccctctacagccctcaggtacctcattgaggagctggtcaacatcacccagaaccagaaggctccgctctgcaatggcagcatggtatggagcatcaacctgacagctggcatgtactgtgcagccctggaatccctgatcaacgtgtcaggctgcagtgccatcgagaagacccagaggatgctgagcggattctgcccgcacaaggtctcagctgggcagttttccagcttgcatgtccgagacaccaaaatcgaggtggcccagtttgtaaaggacctgctcttacatttaaagaaactttttcgcgagggacggttcaacgagtccaaatatggtcccccatgcccaccatgcccagcacctgagttcctggggggaccatcagtcttcctgttccccccaaaacccaaggacactctcatgatctcccggacccctgaggtcacgtgcgtggtggtggacgtgagccaggaagaccccgaggtccagttcaactggtacgtggatggcgtggaggtgcataatgccaagacaaagccgcgggaggagcagttcaacagcacgtaccgtgtggtcagcgtcctcaccgtcctgcaccaggactggctgaacggcaaggagtacaagtgcaaggtctccaacaaaggcctcccgtcctccatcgagaaaaccatctccaaagccaaagggcagccccgagagccacaggtgtacaccctgcccccatcccaggaggagatgaccaagaaccaggtcagcctgacctgcctggtcaaaggcttctaccccagcgacatcgccgtggagtgggagagcaatgggcagccggagaacaactacaagaccacgcctcccgtgctggactccgacggctccttcttcctctacagcaggctaaccgtggacaagagcaggtggcaggaggggaatgtcttctcatgctccgtgatgcatgaggctctgcacaaccactacacacagaagagcctctccctgtctctgggtaaaatggccctgattgtgctggggggcgtcgccggcctcctgcttttcattgggctaggcatcttcttcagagtgaagttcagcaggagcgcagacgcccccgcgtaccagcagggccagaaccagctctataacgagctcaatctaggacgaagagaggagtacgatgttttggacaagagacgtggccgggaccctgagatggggggaaagccgagaaggaagaaccctcaggaaggcctgtacaatgaactgcagaaagataagatggcggaggcctacagtgagattgggatgaaaggcgagcgccggaggggcaaggggcacgatggcctttaccagggtctcagtacagccaccaaggacacctacgacgcccttcacatgcaggccctgccccctcgctaagcggccgcat

SEQ ID NO: 6 - DNA, 1522 bp, Homo sapiens
tagagatctcggcggtggtacgaagaggaccactgttcggaagacgagacactcaatggtgtgggtcgtaaggaggactagggtccgggacacggagggagatgtcgggagtccatggagtaactcctcgaccagttgtagtgggtcttggtcttccgaggcgagacgttaccgtcgtaccatacctcgtagttggactgtcgaccgtacatgacacgtcgggaccttagggactagttgcacagtccgacgtcacggtagctcttctgggtctcctacgactcgcctaagacgggcgtgttccagagtcgacccgtcaaaaggtcgaacgtacaggctctgtggttttagctccaccgggtcaaacatttcctggacgagaatgtaaatttctttgaaaaagcgctccctgccaagttgctcaggtttataccagggggtacgggtggtacgggtcgtggactcaaggacccccctggtagtcagaaggacaaggggggttttgggttcctgtgagagtactagagggcctggggactccagtgcacgcaccaccacctgcactcggtccttctggggctccaggtcaagttgaccatgcacctaccgcacctccacgtattacggttctgtttcggcgccctcctcgtcaagttgtcgtgcatggcacaccagtcgcaggagtggcaggacgtggtcctgaccgacttgccgttcctcatgttcacgttccagaggttgtttccggagggcaggaggtagctcttttggtagaggtttcggtttcccgtcggggctctcggtgtccacatgtgggacgggggtagggtcctcctctactggttcttggtccagtcggactggacggaccagtttccgaagatggggtcgctgtagcggcacctcaccctctcgttacccgtcggcctcttgttgatgttctggtgcggagggcacgacctgaggctgccgaggaagaaggagatgtcgtccgattggcacctgttctcgtccaccgtcctccccttacagaagagtacgaggcactacgtactccgagacgtgttggtgatgtgtgtcttctcggagagggacagagacccattttaccgggactaacacgaccccccgcagcggccggaggacgaaaagtaacccgatccgtagaagaagtctcacttcaagtcgtcctcgcgtctgcgggggcgcatggtcgtcccggtcttggtcgagatattgctcgagttagatcctgcttctctcctcatgctacaaaacctgttctctgcaccggccctgggactctacccccctttcggctcttccttcttgggagtccttccggacatgttacttgacgtctttctattctaccgcctccggatgtcactctaaccctactttccgctcgcggcctccccgttccccgtgctaccggaaatggtcccagagtcatgtcggtggttcctgtggatgctgcgggaagtgtacgtccgggacgggggagcgattcgccggcgta

SEQ ID NO: 7 - DNA, 84 bp, Homo sapiens
atctctagagccgccaccatgcttctcctggtgacaagccttctgctctgtgagttaccacacccagcattcctcctgatccca

SEQ ID NO: 8 - DNA, 336 bp, Homo sapiens
ggccctgtgcctccctctacagccctcaggtacctcattgaggagctggtcaacatcacccagaaccagaaggctccgctctgcaatggcagcatggtatggagcatcaacctgacagctggcatgtactgtgcagccctggaatccctgatcaacgtgtcaggctgcagtgccatcgagaagacccagaggatgctgagcggattctgcccgcacaaggtctcagctgggcagttttccagcttgcatgtccgagacaccaaaatcgaggtggcccagtttgtaaaggacctgctcttacatttaaagaaactttttcgcgagggacggttcaac

SEQ ID NO: 9 - DNA, 686 bp, Homo sapiens
gagtccaaatatggtcccccatgcccaccatgcccagcacctgagttcctggggggaccatcagtcttcctgttccccccaaaacccaaggacactctcatgatctcccggacccctgaggtcacgtgcgtggtggtggacgtgagccaggaagaccccgaggtccagttcaactggtacgtggatggcgtggaggtgcataatgccaagacaaagccgcgggaggagcagttcaacagcacgtaccgtgtggtcagcgtcctcaccgtcctgcaccaggactggctgaacggcaaggagtacaagtgcaaggtctccaacaaaggcctcccgtcctccatcgagaaaaccatctccaaagccaaagggcagccccgagagccacaggtgtacaccctgcccccatcccaggaggagatgaccaagaaccaggtcagcctgacctgcctggtcaaaggcttctaccccagcgacatcgccgtggagtgggagagcaatgggcagccggagaacaactacaagaccacgcctcccgtgctggactccgacggctccttcttcctctacagcaggctaaccgtggacaagagcaggtggcaggaggggaatgtcttctcatgctccgtgatgcatgaggctctgcacaaccactacacacagaagagcctctccctgtctctgggtaa

SEQ ID NO: 10 - DNA, 67 bp, Homo sapiens
aatggccctgattgtgctggggggcgtcgccggcctcctgcttttcattgggctaggcatcttcttc

SEQ ID NO: 11 - DNA, 339 bp, Homo sapiens
agagtgaagttcagcaggagcgcagacgcccccgcgtaccagcagggccagaaccagctctataacgagctcaatctaggacgaagagaggagtacgatgttttggacaagagacgtggccgggaccctgagatggggggaaagccgagaaggaagaaccctcaggaaggcctgtacaatgaactgcagaaagataagatggcggaggcctacagtgagattgggatgaaaggcgagcgccggaggggcaaggggcacgatggcctttaccagggtctcagtacagccaccaaggacacctacgacgcccttcacatgcaggccctgccccctcgctaa

SEQ ID NO: 12 - DNA, 1092 bp, Artificial Sequence
  plasmid vector
gagtccaaatatggtcccccatgcccaccatgcccagcacctgagttcctggggggaccatcagtcttcctgttccccccaaaacccaaggacactctcatgatctcccggacccctgaggtcacgtgcgtggtggtggacgtgagccaggaagaccccgaggtccagttcaactggtacgtggatggcgtggaggtgcataatgccaagacaaagccgcgggaggagcagttcaacagcacgtaccgtgtggtcagcgtcctcaccgtcctgcaccaggactggctgaacggcaaggagtacaagtgcaaggtctccaacaaaggcctcccgtcctccatcgagaaaaccatctccaaagccaaagggcagccccgagagccacaggtgtacaccctgcccccatcccaggaggagatgaccaagaaccaggtcagcctgacctgcctggtcaaaggcttctaccccagcgacatcgccgtggagtgggagagcaatgggcagccggagaacaactacaagaccacgcctcccgtgctggactccgacggctccttcttcctctacagcaggctaaccgtggacaagagcaggtggcaggaggggaatgtcttctcatgctccgtgatgcatgaggctctgcacaaccactacacacagaagagcctctccctgtctctgggtaaaatggccctgattgtgctggggggcgtcgccggcctcctgcttttcattgggctaggcatcttcttcagagtgaagttcagcaggagcgcagacgcccccgcgtaccagcagggccagaaccagctctataacgagctcaatctaggacgaagagaggagtacgatgttttggacaagagacgtggccgggaccctgagatggggggaaagccgagaaggaagaaccctcaggaaggcctgtacaatgaactgcagaaagataagatggcggaggcctacagtgagattgggatgaaaggcgagcgccggaggggcaaggggcacgatggcctttaccagggtctcagtacagccaccaaggacacctacgacgcccttcacatgcaggccctgccccctcgctaa

SEQ ID NO: 13 - DNA, 6770 bp, Artificial Sequence
  plasmid vector
tcgaaggatctgcgatcgctccggtgcccgtcagtgggcagagcgcacatcgcccacagtccccgagaagttggggggaggggtcggcaattgaaccggtgcctagagaaggtggcgcggggtaaactgggaaagtgatgtcgtgtactggctccgcctttttcccgagggtgggggagaaccgtatataagtgcagtagtcgccgtgaacgttctttttcgcaacgggtttgccgccagaacacagctgaagcttcgaggggctcgcatctctccttcacgcgcccgccgccctacctgaggccgccatccacgccggttgagtcgcgttctgccgcctcccgcctgtggtgcctcctgaactgcgtccgccgtctaggtaagtttaaagctcaggtcgagaccgggcctttgtccggcgctcccttggagcctacctagactcagccggctctccacgctttgcctgaccctgcttgctcaactctacgtctttgtttcgttttctgttctgcgccgttacagatccaagctgtgaccggcgcctacgtaagtgatatctactagatttatcaaaaagagtgttgacttgtgagcgctcacaattgatacggattcatcgagagggacacgtcgactactaaccttcttctctttcctacagctgagatcaccctagagccgccaccatgcttctcctggtgacaagccttctgctctgtgagttaccacacccagcattcctcctgatcccaggccctgtgcctccctctacagccctcaggtacctcattgaggagctggtcaacatcacccagaaccagaaggctccgctctgcaatggcagcatggtatggagcatcaacctgacagctggcatgtactgtgcagccctggaatccctgatcaacgtgtcaggctgcagtgccatcgagaagacccagaggatgctgagcggattctgcccgcacaaggtctcagctgggcagttttccagcttgcatgtccgagacaccaaaatcgaggtggcccagtttgtaaaggacctgctcttacatttaaagaaactttttcgcgagggacggttcaacgagtccaaatatggtcccccatgcccaccatgcccagcacctgagttcctggggggaccatcagtcttcctgttccccccaaaacccaaggacactctcatgatctcccggacccctgaggtcacgtgcgtggtggtggacgtgagccaggaagaccccgaggtccagttcaactggtacgtggatggcgtggaggtgcataatgccaagacaaagccgcgggaggagcagttcaacagcacgtaccgtgtggtcagcgtcctcaccgtcctgcaccaggactggctgaacggcaaggagtacaagtgcaaggtctccaacaaaggcctcccgtcctccatcgagaaaaccatctccaaagccaaagggcagccccgagagccacaggtgtacaccctgcccccatcccaggaggagatgaccaagaaccaggtcagcctgacctgcctggtcaaaggcttctaccccagcgacatcgccgtggagtgggagagcaatgggcagccggagaacaactacaagaccacgcctcccgtgctggactccgacggctccttcttcctctacagcaggctaaccgtggacaagagcaggtggcaggaggggaatgtcttctcatgctccgtgatgcatgaggctctgcacaaccactacacacagaagagcctctccctgtccctaggtaaaatggccctgattgtgctggggggcgtcgccggcctcctgcttttcattgggctaggcatcttcttcagagtgaagttcagcaggagcgcagacgcccccgcgtaccagcagggccagaaccagctctataacgagctcaatctaggacgaagagaggagtacgatgttttggacaagagacgtggccgggaccctgagatggggggaaagccgagaaggaagaaccctcaggaaggcctgtacaatgaactgcagaaagataagatggcggaggcctacagtgagattgggatgaaaggcgagcgccggaggggcaaggggcacgatggcctttaccagggtctcagtacagccaccaaggacacctacgacgcccttcacatgcaggccctgccccctcgctgagcggccggcgaaggaggcctagatctatcgattgtacagctagctcgacatgataagatacattgatgagtttggacaaaccacaactagaatgcagtgaaaaaaatgctttatttgtgaaatttgtgatgctattgctttatttgtgaaatttgtgatgctattgctttatttgtaaccattataagctgcaataaacaagttaacaacaacaattgcattcattttatgtttcaggttcagggggaggtgtgggaggttttttaaagcaagtaaaacctctacaaatgtggtagatccatttaaatgttagcgaagaacatgtgagcaaaaggccagcaaaaggccaggaaccgtaaaaaggccgcgttgctggcgtttttccataggctccgcccccctgacgagcatcacaaaaatcgacgctcaagtcagaggtggcgaaacccgacaggactataaagataccaggcgtttccccctggaagctccctcgtgcgctctcctgttccgaccctgccgcttaccggatacctgtccgcctttctcccttcgggaagcgtggcgctttctcaatgctcacgctgtaggtatctcagttcggtgtaggtcgttcgctccaagctgggctgtgtgcacgaaccccccgttcagcccgaccgctgcgccttatccggtaactatcgtcttgagtccaacccggtaagacacgacttatcgccactggcagcagccactggtaacaggattagcagagcgaggtatgtaggcggtgctacagagttcttgaagtggtggcctaactacggctacactagaagaacagtatttggtatctgcgctctgctgaagccagttaccttcggaaaaagagttggtagctcttgatccggcaaacaaaccaccgctggtagcggtggtttttttgtttgcaagcagcagattacgcgcagaaaaaaaggatctcaagaagatcctttgatcttttctacggggtctgacgctcagtggaacgaaaactcacgttaagggattttggtcatggctagttaattaagctgcaataaacaatcattattttcattggatctgtgtgttggttttttgtgtgggcttgggggagggggaggccagaatgactccaagagctacaggaaggcaggtcagagaccccactggacaaacagtggctggactctgcaccataacacacaatcaacaggggagtgagctggatcgagctagagtccgttacataacttacggtaaatggcccgcctggctgaccgcccaacgacccccgcccattgacgtcaataatgacgtatgttcccatagtaacgccaatagggactttccattgacgtcaatgggtggagtatttacggtaaactgcccacttggcagtacatcaagtgtatcatatgccaagtacgccccctattgacgtcaatgacggtaaatggcccgcctggcattatgcccagtacatgaccttatgggactttcctacttggcagtacatctacgtattagtcatcgctattaccatggtgatgcggttttggcagtacatcaatgggcgtggatagcggtttgactcacggggatttccaagtctccaccccattgacgtcaatgggagtttgttttggcaccaaaatcaacgggactttccaaaatgtcgtaacaactccgccccattgacgcaaatgggcggtaggcgtgtacggtgggaggtctatataagcagagctcgtttagtgaaccgtcagatcgcctggagacgccatccacgctgttttgacctccatagaagacaccgggaccgatccagcctccgcggccgggaacggtgcattggaacgcggattccccgtgccaagagtgacgtaagtaccgcctatagagtctataggcccacctagttgtgaccggcgcctagtgttgacaattaatcatcggcatagtataatacgactcactataggagggccaccatgtcgactactaaccttcttctctttcctacagctgagatcaccggtaggagggccatcatgaaaaagcctgaactcaccgcgacgtctgtcgcgaagtttctgatcgaaaagttcgacagcgtctccgacctgatgcagctctcggagggcgaagaatctcgtgctttcagcttcgatgtaggagggcgtggatatgtcctgcgggtaaatagctgcgccgatggtttctacaaagatcgttatgtttatcggcactttgcatcggccgcgctcccgattccggaagtgcttgacattggggaattcagcgagagcctgacctattgcatctcccgccgtgcacagggtgtcacgttgcaagacctgcctgaaaccgaactgcccgctgttctgcaacccgtcgcggagctcatggatgcgatcgctgcggccgatcttagccagacgagcgggttcggcccattcggaccgcaaggaatcggtcaatacactacatggcgtgatttcatatgcgcgattgctgatccccatgtgtatcactggcaaactgtgatggacgacaccgtcagtgcgtccgtcgcgcaggctctcgatgagctgatgctttgggccgaggactgccccgaagtccggcacctcgtgcacgcggatttcggctccaacaatgtcctgacggacaatggccgcataacagcggtcattgactggagcgaggcgatgttcggggattcccaatacgaggtcgccaacatcttcttctggaggccgtggttggcttgtatggagcagcagacgcgctacttcgagcggaggcatccggagcttgcaggatcgccgcggctccgggcgtatatgctccgcattggtcttgaccaactctatcagagcttggttgacggcaatttcgatgatgcagcttgggcgcagggtcgatgcgacgcaatcgtccgatccggagccgggactgtcgggcgtacacaaatcgcccgcagaagcgcggccgtctggaccgatggctgtgtagaagtcgcgtctgcgttcgaccaggctgcgcgttctcgcggccatagcaaccgacgtacggcgttgcgccctcgccggcagcaagaagccacggaagtccgcccggagcagaaaatgcccacgctactgcgggtttatatagacggtccccacgggatggggaaaaccaccaccacgcaactgctggtggccctgggttcgcgcgacgatatcgtctacgtacccgagccgatgacttactggcgggtgctgggggcttccgagacaatcgcgaacatctacaccacacaacaccgcctcgaccagggtgagatatcggccggggacgcggcggtggtaatgacaagcgcccagataacaatgggcatgccttatgccgtgaccgacgccgttctggctcctcatatcgggggggaggctgggagctcacatgccccgcccccggccctcaccctcatcttcgaccgccatcccatcgccgccctcctgtgctacccggccgcgcggtaccttatgggcagcatgaccccccaggccgtgctggcgttcgtggccctcatcccgccgaccttgcccggcaccaacatcgtgcttggggcccttccggaggacagacacatcgaccgcctggccaaacgccagcgccccggcgagcggctggacctggctatgctggctgcgattcgccgcgtttacgggctacttgccaatacggtgcggtatctgcagtgcggcgggtcgtggcgggaggactggggacagctttcggggacggccgtgccgccccagggtgccgagccccagagcaacgcgggcccacgaccccatatcggggacacgttatttaccctgtttcgggcccccgagttgctggcccccaacggcgacctgtataacgtgtttgcctgggccttggacgtcttggccaaacgcctccgttccatgcacgtctttatcctggattacgaccaatcgcccgccggctgccgggacgccctgctgcaacttacctccgggatggtccagacccacgtcaccacccccggctccataccgacgatatgcgacctggcgcgcacgtttgcccgggagatgggggaggctaactgagtcgagaattcgctagagggccctattctatagtgtcacctaaatgctagagctcgctgatcagcctcgactgtgccttctagttgccagccatctgttgtttgcccctcccccgtgccttccttgaccctggaaggtgccactcccactgtcctttcctaataaaatgaggaaattgcatcgcattgtctgagtaggtgtcattctattctggggggtggggtggggcaggacagcaagggggaggattgggaagacaatagcaggcatgcgcagggcccaattgctcgagcggccgcaataaaatatctttattttcattacatctgtgtgttggttttttgtgtgaatcgtaactaacatacgctctccatcaaaacaaaacgaaacaaaacaaactagcaaaataggctgtccccagtgcaagtgcaggtgccagaacatttctcta

SEQ ID NO: 14 - DNA, 6770 bp, Homo sapiens
agcttcctagacgctagcgaggccacgggcagtcacccgtctcgcgtgtagcgggtgtcaggggctcttcaacccccctccccagccgttaacttggccacggatctcttccaccgcgccccatttgaccctttcactacagcacatgaccgaggcggaaaaagggctcccaccccctcttggcatatattcacgtcatcagcggcacttgcaagaaaaagcgttgcccaaacggcggtcttgtgtcgacttcgaagctccccgagcgtagagaggaagtgcgcgggcggcgggatggactccggcggtaggtgcggccaactcagcgcaagacggcggagggcggacaccacggaggacttgacgcaggcggcagatccattcaaatttcgagtccagctctggcccggaaacaggccgcgagggaacctcggatggatctgagtcggccgagaggtgcgaaacggactgggacgaacgagttgagatgcagaaacaaagcaaaagacaagacgcggcaatgtctaggttcgacactggccgcggatgcattcactatagatgatctaaatagtttttctcacaactgaacactcgcgagtgttaactatgcctaagtagctctccctgtgcagctgatgattggaagaagagaaaggatgtcgactctagtgggatctcggcggtggtacgaagaggaccactgttcggaagacgagacactcaatggtgtgggtcgtaaggaggactagggtccgggacacggagggagatgtcgggagtccatggagtaactcctcgaccagttgtagtgggtcttggtcttccgaggcgagacgttaccgtcgtaccatacctcgtagttggactgtcgaccgtacatgacacgtcgggaccttagggactagttgcacagtccgacgtcacggtagctcttctgggtctcctacgactcgcctaagacgggcgtgttccagagtcgacccgtcaaaaggtcgaacgtacaggctctgtggttttagctccaccgggtcaaacatttcctggacgagaatgtaaatttctttgaaaaagcgctccctgccaagttgctcaggtttataccagggggtacgggtggtacgggtcgtggactcaaggacccccctggtagtcagaaggacaaggggggttttgggttcctgtgagagtactagagggcctggggactccagtgcacgcaccaccacctgcactcggtccttctggggctccaggtcaagttgaccatgcacctaccgcacctccacgtattacggttctgtttcggcgccctcctcgtcaagttgtcgtgcatggcacaccagtcgcaggagtggcaggacgtggtcctgaccgacttgccgttcctcatgttcacgttccagaggttgtttccggagggcaggaggtagctcttttggtagaggtttcggtttcccgtcggggctctcggtgtccacatgtgggacgggggtagggtcctcctctactggttcttggtccagtcggactggacggaccagtttccgaagatggggtcgctgtagcggcacctcaccctctcgttacccgtcggcctcttgttgatgttctggtgcggagggcacgacctgaggctgccgaggaagaaggagatgtcgtccgattggcacctgttctcgtccaccgtcctccccttacagaagagtacgaggcactacgtactccgagacgtgttggtgatgtgtgtcttctcggagagggacagggatccattttaccgggactaacacgaccccccgcagcggccggaggacgaaaagtaacccgatccgtagaagaagtctcacttcaagtcgtcctcgcgtctgcgggggcgcatggtcgtcccggtcttggtcgagatattgctcgagttagatcctgcttctctcctcatgctacaaaacctgttctctgcaccggccctgggactctacccccctttcggctcttccttcttgggagtccttccggacatgttacttgacgtctttctattctaccgcctccggatgtcactctaaccctactttccgctcgcggcctccccgttccccgtgctaccggaaatggtcccagagtcatgtcggtggttcctgtggatgctgcgggaagtgtacgtccgggacgggggagcgactcgccggccgcttcctccggatctagatagctaacatgtcgatcgagctgtactattctatgtaactactcaaacctgtttggtgttgatcttacgtcactttttttacgaaataaacactttaaacactacgataacgaaataaacactttaaacactacgataacgaaataaacattggtaatattcgacgttatttgttcaattgttgttgttaacgtaagtaaaatacaaagtccaagtccccctccacaccctccaaaaaatttcgttcattttggagatgtttacaccatctaggtaaatttacaatcgcttcttgtacactcgttttccggtcgttttccggtccttggcatttttccggcgcaacgaccgcaaaaaggtatccgaggcggggggactgctcgtagtgtttttagctgcgagttcagtctccaccgctttgggctgtcctgatatttctatggtccgcaaagggggaccttcgagggagcacgcgagaggacaaggctgggacggcgaatggcctatggacaggcggaaagagggaagcccttcgcaccgcgaaagagttacgagtgcgacatccatagagtcaagccacatccagcaagcgaggttcgacccgacacacgtgcttggggggcaagtcgggctggcgacgcggaataggccattgatagcagaactcaggttgggccattctgtgctgaatagcggtgaccgtcgtcggtgaccattgtcctaatcgtctcgctccatacatccgccacgatgtctcaagaacttcaccaccggattgatgccgatgtgatcttcttgtcataaaccatagacgcgagacgacttcggtcaatggaagcctttttctcaaccatcgagaactaggccgtttgtttggtggcgaccatcgccaccaaaaaaacaaacgttcgtcgtctaatgcgcgtctttttttcctagagttcttctaggaaactagaaaagatgccccagactgcgagtcaccttgcttttgagtgcaattccctaaaaccagtaccgatcaattaattcgacgttatttgttagtaataaaagtaacctagacacacaaccaaaaaacacacccgaaccccctccccctccggtcttactgaggttctcgatgtccttccgtccagtctctggggtgacctgtttgtcaccgacctgagacgtggtattgtgtgttagttgtcccctcactcgacctagctcgatctcaggcaatgtattgaatgccatttaccgggcggaccgactggcgggttgctgggggcgggtaactgcagttattactgcatacaagggtatcattgcggttatccctgaaaggtaactgcagttacccacctcataaatgccatttgacgggtgaaccgtcatgtagttcacatagtatacggttcatgcgggggataactgcagttactgccatttaccgggcggaccgtaatacgggtcatgtactggaataccctgaaaggatgaaccgtcatgtagatgcataatcagtagcgataatggtaccactacgccaaaaccgtcatgtagttacccgcacctatcgccaaactgagtgcccctaaaggttcagaggtggggtaactgcagttaccctcaaacaaaaccgtggttttagttgccctgaaaggttttacagcattgttgaggcggggtaactgcgtttacccgccatccgcacatgccaccctccagatatattcgtctcgagcaaatcacttggcagtctagcggacctctgcggtaggtgcgacaaaactggaggtatcttctgtggccctggctaggtcggaggcgccggcccttgccacgtaaccttgcgcctaaggggcacggttctcactgcattcatggcggatatctcagatatccgggtggatcaacactggccgcggatcacaactgttaattagtagccgtatcatattatgctgagtgatatcctcccggtggtacagctgatgattggaagaagagaaaggatgtcgactctagtggccatcctcccggtagtactttttcggacttgagtggcgctgcagacagcgcttcaaagactagcttttcaagctgtcgcagaggctggactacgtcgagagcctcccgcttcttagagcacgaaagtcgaagctacatcctcccgcacctatacaggacgcccatttatcgacgcggctaccaaagatgtttctagcaatacaaatagccgtgaaacgtagccggcgcgagggctaaggccttcacgaactgtaaccccttaagtcgctctcggactggataacgtagagggcggcacgtgtcccacagtgcaacgttctggacggactttggcttgacgggcgacaagacgttgggcagcgcctcgagtacctacgctagcgacgccggctagaatcggtctgctcgcccaagccgggtaagcctggcgttccttagccagttatgtgatgtaccgcactaaagtatacgcgctaacgactaggggtacacatagtgaccgtttgacactacctgctgtggcagtcacgcaggcagcgcgtccgagagctactcgactacgaaacccggctcctgacggggcttcaggccgtggagcacgtgcgcctaaagccgaggttgttacaggactgcctgttaccggcgtattgtcgccagtaactgacctcgctccgctacaagcccctaagggttatgctccagcggttgtagaagaagacctccggcaccaaccgaacatacctcgtcgtctgcgcgatgaagctcgcctccgtaggcctcgaacgtcctagcggcgccgaggcccgcatatacgaggcgtaaccagaactggttgagatagtctcgaaccaactgccgttaaagctactacgtcgaacccgcgtcccagctacgctgcgttagcaggctaggcctcggccctgacagcccgcatgtgtttagcgggcgtcttcgcgccggcagacctggctaccgacacatcttcagcgcagacgcaagctggtccgacgcgcaagagcgccggtatcgttggctgcatgccgcaacgcgggagcggccgtcgttcttcggtgccttcaggcgggcctcgtcttttacgggtgcgatgacgcccaaatatatctgccaggggtgccctaccccttttggtggtggtgcgttgacgaccaccgggacccaagcgcgctgctatagcagatgcatgggctcggctactgaatgaccgcccacgacccccgaaggctctgttagcgcttgtagatgtggtgtgttgtggcggagctggtcccactctatagccggcccctgcgccgccaccattactgttcgcgggtctattgttacccgtacggaatacggcactggctgcggcaagaccgaggagtatagccccccctccgaccctcgagtgtacggggcgggggccgggagtgggagtagaagctggcggtagggtagcggcgggaggacacgatgggccggcgcgccatggaatacccgtcgtactggggggtccggcacgaccgcaagcaccgggagtagggcggctggaacgggccgtggttgtagcacgaaccccgggaaggcctcctgtctgtgtagctggcggaccggtttgcggtcgcggggccgctcgccgacctggaccgatacgaccgacgctaagcggcgcaaatgcccgatgaacggttatgccacgccatagacgtcacgccgcccagcaccgccctcctgacccctgtcgaaagcccctgccggcacggcggggtcccacggctcggggtctcgttgcgcccgggtgctggggtatagcccctgtgcaataaatgggacaaagcccgggggctcaacgaccgggggttgccgctggacatattgcacaaacggacccggaacctgcagaaccggtttgcggaggcaaggtacgtgcagaaataggacctaatgctggttagcgggcggccgacggccctgcgggacgacgttgaatggaggccctaccaggtctgggtgcagtggtgggggccgaggtatggctgctatacgctggaccgcgcgtgcaaacgggccctctaccccctccgattgactcagctcttaagcgatctcccgggataagatatcacagtggatttacgatctcgagcgactagtcggagctgacacggaagatcaacggtcggtagacaacaaacggggagggggcacggaaggaactgggaccttccacggtgagggtgacaggaaaggattattttactcctttaacgtagcgtaacagactcatccacagtaagataagaccccccaccccaccccgtcctgtcgttccccctcctaacccttctgttatcgtccgtacgcgtcccgggttaacgagctcgccggcgttattttatagaaataaaagtaatgtagacacacaaccaaaaaacacacttagcattgattgtatgcgagaggtagttttgttttgctttgttttgtttgatcgttttatccgacaggggtcacgttcacgtccacggtcttgtaaagagat

SEQ ID NO: 15 - protein, 497 aa, Homo sapiens; identical to SEQ ID NO: 4

SEQ ID NO: 16 - protein, 691 aa, Homo sapiens
MKKPELTATSVAKFLIEKFDSVSDLMQLSEGEESRAFSFDVGGRGYVLRVNSCADGFYKDRYVYRHFASAALPIPEVLDIGEFSESLTYCISRRAQGVTLQDLPETELPAVLQPVAELMDAIAAADLSQTSGFGPFGPQGIGQYTTWRDFICAIADPHVYHWQTVMDDTVSASVAQALDELMLWAEDCPEVRHLVHADFGSNNVLTDNGRITAVIDWSEAMFGDSQYEVANIFFWRPWLACMEQQTRYFERRHPELAGSPRLRAYMLRIGLDQLYQSLVDGNFDDAAWAQGRCDAIVRSGAGTVGRTQIARRSAAVWTDGCVEVASAFDQAARSRGHSNRRTALRPRRQQEATEVRPEQKMPTLLRVYIDGPHGMGKTTTTQLLVALGSRDDIVYVPEPMTYWRVLGASETIANIYTTQHRLDQGEISAGDAAVVMTSAQITMGMPYAVTDAVLAPHIGGEAGSSHAPPPALTLIFDRHPIAALLCYPAARYLMGSMTPQAVLAFVALIPPTLPGTNIVLGALPEDRHIDRLAKRQRPGERLDLAMLAAIRRVYGLLANTVRYLQCGGSWREDWGQLSGTAVPPQGAEPQSNAGPRPHIGDTLFTLFRAPELLAPNGDLYNVFAWALDVLAKRLRSMHVFILDYDQSPAGCRDALLQLTSGMVQTHVTTPGSIPTICDLARTFAREMGEAN

SEQ ID NO: 17 - DNA, 102 bp, Homo sapiens
tatgaattcatggcgcttttgttgaccacggtcattgctctcacttgccttggcggctttgcctccccaggccctgtgcctccctctacagccctcaggtac

SEQ ID NO: 18 - DNA, 101 bp, Homo sapiens
gttgatgctccataccatgctgccattgcagagcggagccttctggttctgggtgatgttgaccagctcctcaatgaggtacctgagggctgtagagggag

SEQ ID NO: 19 - DNA, 100 bp, Homo sapiens
ctctgggtcttctcgatggcactgcagcctgacacgttgatcagggattccagggctgcacagtacatgccagctgtcaggttgatgctccataccatgc

SEQ ID NO: 20 - DNA, 100 bp, Homo sapiens
cctcgattttggtgtctcggacatgcaagctggaaaactgcccagctgagaccttgtgcgggcagaatccgctcagcatcctctgggtcttctcgatggc

SEQ ID NO: 21 - DNA, 96 bp, Homo sapiens
tcggatcctcagttgaaccgtccctcgcgaaaaagtttctttaaatgtaagagcaggtcctttacaaactgggccacctcgattttggtgtctcgg

SEQ ID NO: 22 - DNA, 39 bp, Homo sapiens
caacctgacagctggcatgtactgtgcagccctggaatc

SEQ ID NO: 23 - DNA, 39 bp, Homo sapiens
gttggactgtcgaccgtacatgacacgtcgggaccttag

SEQ ID NO: 24 - DNA, 43 bp, Homo sapiens
atctctagagccgccaccatgcttctcctggtgacaagccttc

SEQ ID NO: 25 - DNA, 34 bp, Homo sapiens
gagggaggcacagggcctgggatcaggaggaatg

SEQ ID NO: 26 - DNA, 34 bp, Homo sapiens
cattcctcctgatcccaggccctgtgcctccctc

SEQ ID NO: 27 - DNA, 35 bp, Homo sapiens
gggaccatatttggactcgttgaaccgtccctcgc

SEQ ID NO: 28 - DNA, 35 bp, Homo sapiens
gcgagggacggttcaacgagtccaaatatggtccc

SEQ ID NO: 29 - DNA, 26 bp, Homo sapiens
atgcggccgctcagcgagggggcagg

SEQ ID NO: 30 - DNA, 39 bp, Homo sapiens
atcgaattcgccgccaccatgggaaacagctgttacaac

SEQ ID NO: 31 - DNA, 36 bp, Homo sapiens
gataagcttatcgattcaccacatcctccttcagtt

SEQ ID NO: 32 - DNA, 43 bp, Homo sapiens
cattgggctaggcatcttcttcaggagtaagaggagcaggctc

SEQ ID NO: 33 - DNA, 47 bp, Homo sapiens
gtttctttctgccccgtttgccacctccggagcgataggctgcgaag

SEQ ID NO: 34 - DNA, 47 bp, Homo sapiens
cttcgcagcctatcgctccggaggtggcaaacggggcagaaagaaac

SEQ ID NO: 35 - DNA, 38 bp, Homo sapiens
gttgcggccgctcacagttcacatcctccttcttcttc

SEQ ID NO: 36 - DNA, 1644 bp, Homo sapiens
atgctgctgctggtgaccagcctgctgctgtgcgagctgccccaccccgcctttctgctgatccctggccccgtgccccctagcaccgccctgcgctacctgatcgaggaactggtgaacatcacccagaaccagaaagcccccctgtgcaacggcagcatggtgtggagcatcaacctgaccgccggcatgtactgtgccgccctggaaagcctgatcaacgtgagcggctgcagcgccatcgagaaaacccagcggatgctgtccggcttctgcccccacaaggtgtccgccggacagttcagcagcctgcacgtgcgggacaccaagatcgaggtggcccagttcgtgaaggacctgctgctgcacctgaagaagctgttccgggagggccggttcaacgagagcaagtacggccctccctgccccccttgccctgccccagagttcctgggcggacccagcgtgttcctgttcccccccaagcccaaggacaccctgatgatcagccggacccctgaggtgacctgcgtggtggtggacgtgagccaggaagatcctgaggtccagttcaattggtacgtggacggcgtggaagtgcacaacgccaagaccaagcccagagaggaacagttcaacagcacctaccgggtggtgtctgtgctgaccgtgctgcaccaggactggctgaacggcaaagaatacaagtgcaaggtgtccaacaagggcctgcccagcagcatcgaaaagaccatcagcaaggccaagggccagcctcgcgagccccaggtgtacaccctgcctccctcccaggaagagatgaccaagaaccaggtgtccctgacctgcctggtgaagggcttctaccccagcgacatcgccgtggagtgggagagcaacggccagcctgagaacaactacaagaccacccctcccgtgctggacagcgacggcagcttcttcctgtacagccggctgaccgtggacaagagccggtggcaggaaggcaacgtctttagctgcagcgtgatgcacgaggccctgcacaaccactacacccagaagagcctgagcctgtccctgggcaagatgttctgggtgctggtggtggtgggcggggtgctggcctgctacagcctgctggtgacagtggccttcatcatcttttgggtgcggagcaagcggagcagaggcggccacagcgactacatgaacatgacccccagacggcctggccccacccggaagcactaccagccctacgccccacccagggactttgccgcctaccggtccggcggagggcgggtgaagttcagcagaagcgccgacgcccctgcctaccagcagggccagaatcagctgtacaacgagctgaacctgggcagaagggaagagtacgacgtcctggataagcggagaggccgggaccctgagatgggcggcaagcctcggcggaagaacccccaggaaggcctgtataacgaactgcagaaagacaagatggccgaggcctacagcgagatcggcatgaagggcgagcggaggcggggcaagggccacgacggcctgtatcagggcctgtccaccgccaccaaggatacctacgacgccctgcacatgcaggccctgcccccaaggtga

SEQ ID NO: 37 - DNA, 1761 bp, Homo sapiens
atgcttctcctggtgacaagccttctgctctgtgagttaccacacccagcattcctcctgatcccaggccctgtgcctccctctacagccctcagggagctcattgaggagctggtcaacatcacccagaaccagaaggctccgctctgcaatggcagcatggtatggagcatcaacctgacagctggcatgtactgtgcagccctggaatccctgatcaacgtgtcaggctgcagtgccatcgagaagacccagaggatgctgagcggattctgcccgcacaaggtctcagctgggcagttttccagcttgcatgtccgagacaccaaaatcgaggtggcccagtttgtaaaggacctgctcttacatttaaagaaactttttcgcgagggacggttcaacgagtccaaatatggtcccccatgcccaccatgcccagcacctgagttcctggggggaccatcagtcttcctgttccccccaaaacccaaggacactctcatgatctcccggacccctgaggtcacgtgcgtggtggtggacgtgagccaggaagaccccgaggtccagttcaactggtacgtggatggcgtggaggtgcataatgccaagacaaagccgcgggaggagcagttcaacagcacgtaccgtgtggtcagcgtcctcaccgtcctgcaccaggactggctgaacggcaaggagtacaagtgcaaggtctccaacaaaggcctcccgtcctccatcgagaaaaccatctccaaagccaaagggcagccccgagagccacaggtgtacaccctgcccccatcccaggaggagatgaccaagaaccaggtcagcctgacctgcctggtcaaaggcttctaccccagcgacatcgccgtggagtgggagagcaatgggcagccggagaacaactacaagaccacgcctcccgtgctggactccgacggctccttcttcctctacagcaggctaaccgtggacaagagcaggtggcaggaggggaatgtcttctcatgctccgtgatgcatgaggctctgcacaaccactacacacagaagagcctctccctgtctctgggtaaaatggccctgattgtgctggggggcgtcgccggcctcctgcttttcattgggctaggcatcttcttcaggagtaagaggagcaggctcctgcacagtgactacatgaacatgactccccgccgccctgggcccacccgcaagcattaccagccctatgccccaccacgcgacttcgcagcctatcgctccggaggtggcaaacggggcagaaagaaactcctgtatatattcaaacaaccatttatgagaccagtacaaactactcaagaggaagatggctgtagctgccgatttccagaagaagaagaaggaggatgtgaactgggaggtggcagagtgaagttcagcaggagcgcagacgcccccgcgtaccagcagggccagaaccagctctataacgagctcaatctaggacgaagagaggagtacgatgttttggacaagagacgtggccgggaccctgagatggggggaaagccgagaaggaagaaccctcaggaaggcctgtacaatgaactgcagaaagataagatggcggaggcctacagtgagattgggatgaaaggcgagcgccggaggggcaaggggcacgatggcctttaccagggtctcagtacagccaccaaggacacctacgacgcccttcacatgcaggccctgccccctcgctga

SEQ ID NO: 38 - DNA, 1740 bp, Homo sapiens
atgcttctcctggtgacaagccttctgctctgtgagttaccacacccagcattcctcctgatcccaggccctgtgcctccctctacagccctcaggtacctcattgaggagctggtcaacatcacccagaaccagaaggctccgctctgcaatggcagcatggtatggagcatcaacctgacagctggcatgtactgtgcagccctggaatccctgatcaacgtgtcaggctgcagtgccatcgagaagacccagaggatgctgagcggattctgcccgcacaaggtctcagctgggcagttttccagcttgcatgtccgagacaccaaaatcgaggtggcccagtttgtaaaggacctgctcttacatttaaagaaactttttcgcgagggacggttcaacgagtccaaatatggtcccccatgcccaccatgcccagcacctgagttcctggggggaccatcagtcttcctgttccccccaaaacccaaggacactctcatgatctcccggacccctgaggtcacgtgcgtggtggtggacgtgagccaggaagaccccgaggtccagttcaactggtacgtggatggcgtggaggtgcataatgccaagacaaagccgcgggaggagcagttcaacagcacgtaccgtgtggtcagcgtcctcaccgtcctgcaccaggactggctgaacggcaaggagtacaagtgcaaggtctccaacaaaggcctcccgtcctccatcgagaaaaccatctccaaagccaaagggcagccccgagagccacaggtgtacaccctgcccccatcccaggaggagatgaccaagaaccaggtcagcctgacctgcctggtcaaaggcttctaccccagcgacatcgccgtggagtgggagagcaatgggcagccggagaacaactacaagaccacgcctcccgtgctggactccgacggctccttcttcctctacagcaggctaaccgtggacaagagcaggtggcaggaggggaatgtcttctcatgctccgtgatgcatgaggctctgcacaaccactacacacagaagagcctctccctgtccctaggtaaattttgggtgctggtggtggttggtggagtcctggcttgctatagcttgctagtaacagtggcctttattattttctgggtgaggagtaagaggagcaggctcctgcacagtgactacatgaacatgactccccgccgccccgggcccacccgcaagcattaccagccctatgccccaccacgcgacttcgcagcctatcgctccagggaccagaggctgccccccgatgcccacaagccccctgggggaggcagtttccggacccccatccaagaggagcaggccgacgcccactccaccctggccaagatcagagtgaagttcagcaggagcgcagacgcccccgcgtaccagcagggccagaaccagctctataacgagctcaatctaggacgaagagaggagtacgatgttttggacaagagacgtggccgggaccctgagatggggggaaagccgagaaggaagaaccctcaggaaggcctgtacaatgaactgcagaaagataagatggcggaggcctacagtgagattgggatgaaaggcgagcgccggaggggcaaggggcacgatggcctttaccagggtctcagtacagccaccaaggacacctacgacgcccttcacatgcaggccctgccccctcgctga

SEQ ID NO: 39 - DNA, 1779 bp, Homo sapiens
atgcttctcctggtgacaagccttctgctctgtgagttaccacacccagcattcctcctgatcccaggccctgtgcctccctctacagccctcaggtacctcattgaggagctggtcaacatcacccagaaccagaaggctccgctctgcaatggcagcatggtatggagcatcaacctgacagctggcatgtactgtgcagccctggaatccctgatcaacgtgtcaggctgcagtgccatcgagaagacccagaggatgctgagcggattctgcccgcacaaggtctcagctgggcagttttccagcttgcatgtccgagacaccaaaatcgaggtggcccagtttgtaaaggacctgctcttacatttaaagaaactttttcgcgagggacggttcaacgagtccaaatatggtcccccatgcccaccatgcccagcacctgagttcctggggggaccatcagtcttcctgttccccccaaaacccaaggacactctcatgatctcccggacccctgaggtcacgtgcgtggtggtggacgtgagccaggaagaccccgaggtccagttcaactggtacgtggatggcgtggaggtgcataatgccaagacaaagccgcgggaggagcagttcaacagcacgtaccgtgtggtcagcgtcctcaccgtcctgcaccaggactggctgaacggcaaggagtacaagtgcaaggtctccaacaaaggcctcccgtcctccatcgagaaaaccatctccaaagccaaagggcagccccgagagccacaggtgtacaccctgcccccatcccaggaggagatgaccaagaaccaggtcagcctgacctgcctggtcaaaggcttctaccccagcgacatcgccgtggagtgggagagcaatgggcagccggagaacaactacaagaccacgcctcccgtgctggactccgacggctccttcttcctctacagcaggctaaccgtggacaagagcaggtggcaggaggggaatgtcttctcatgctccgtgatgcatgaggctctgcacaaccactacacacagaagagcctctccctgtccctaggtaaaatgttttgggtgctggtggtggttggtggagtcctggcttgctatagcttgctagtaacagtggcctttattattttctgggtgaggagtaagaggagcaggggcggacacagtgactacatgaacatgactccccgccgccctgggcccacccgcaagcattaccagccctatgccccaccacgcgacttcgcagcctatcgctccggaggtggcaaacggggcagaaagaaactcctgtatatattcaaacaaccatttatgagaccagtacaaactactcaagaggaagatggctgtagctgccgatttccagaagaagaagaaggaggatgtgaactgggaggtggcagagtgaagttcagcaggagcgcagacgcccccgcgtaccagcagggccagaaccagctctataacgagctcaatctaggacgaagagaggagtacgatgttttggacaagagacgtggccgggaccctgagatggggggaaagccgagaaggaagaaccctcaggaaggcctgtacaatgaactgcagaaagataagatggcggaggcctacagtgagattgggatgaaaggcgagcgccggaggggcaaggggcacgatggcctttaccagggtctcagtacagccaccaaggacacctacgacgcccttcacatgcaggccctgccccctcgctga

SEQ ID NO: 40 - DNA, 1779 bp, Homo sapiens
atgcttctcctggtgacaagccttctgctctgtgagttaccacacccagcattcctcctgatcccaggccctgtgcctccctctacagccctcaggtacctcattgaggagctggtcaacatcacccagaaccagaaggctccgctctgcaatggcagcatggtatggagcatcaacctgacagctggcatgtactgtgcagccctggaatccctgatcaacgtgtcaggctgcagtgccatcgagaagacccagaggatgctgagcggattctgcccgcacaaggtctcagctgggcagttttccagcttgcatgtccgagacaccaaaatcgaggtggcccagtttgtaaaggacctgctcttacatttaaagaaactttttcgcgagggacggttcaacgagtccaaatatggtcccccatgcccaccatgcccagcacctgagttcctggggggaccatcagtcttcctgttccccccaaaacccaaggacactctcatgatctcccggacccctgaggtcacgtgcgtggtggtggacgtgagccaggaagaccccgaggtccagttcaactggtacgtggatggcgtggaggtgcataatgccaagacaaagccgcgggaggagcagttcaacagcacgtaccgtgtggtcagcgtcctcaccgtcctgcaccaggactggctgaacggcaaggagtacaagtgcaaggtctccaacaaaggcctcccgtcctccatcgagaaaaccatctccaaagccaaagggcagccccgagagccacaggtgtacaccctgcccccatcccaggaggagatgaccaagaaccaggtcagcctgacctgcctggtcaaaggcttctaccccagcgacatcgccgtggagtgggagagcaatgggcagccggagaacaactacaagaccacgcctcccgtgctggactccgacggctccttcttcctctacagcaggctaaccgtggacaagagcaggtggcaggaggggaatgtcttctcatgctccgtgatgcatgaggctctgcacaaccactacacacagaagagcctctccctgtccctaggtaaaatgttttgggtgctggtggtggttggtggagtcctggcttgctatagcttgctagtaacagtggcctttattattttctgggtgaggagtaagaggagcaggggcggacacagtgactacatgaacatgactccccgccgccctgggcccacccgcaagcattaccagccctatgccccaccacgcgacttcgcagccggaggtggcggaggtggcaaacggggcagaaagaaactcctgtatatattcaaacaaccatttatgagaccagtacaaactactcaagaggaagatggctgtagctgccgatttccagaagaagaagaaggaggatgtgaactgggaggtggcagagtgaagttcagcaggagcgcagacgcccccgcgtaccagcagggccagaaccagctctataacgagctcaatctaggacgaagagaggagtacgatgttttggacaagagacgtggccgggaccctgagatggggggaaagccgagaaggaagaaccctcaggaaggcctgtacaatgaactgcagaaagataagatggcggaggcctacagtgagattgggatgaaaggcgagcgccggaggggcaaggggcacgatggcctttaccagggtctcagtacagccaccaaggacacctacgacgcccttcacatgcaggccctgccccctcgctga

SEQ ID NO: 41 - DNA, 544 bp, Homo sapiens
ggatctgcgatcgctccggtgcccgtcagtgggcagagcgcacatcgcccacagtccccgagaagttggggggaggggtcggcaattgaaccggtgcctagagaaggtggcgcggggtaaactgggaaagtgatgtcgtgtactggctccgcctttttcccgagggtgggggagaaccgtatataagtgcagtagtcgccgtgaacgttctttttcgcaacgggtttgccgccagaacacagctgaagcttcgaggggctcgcatctctccttcacgcgcccgccgccctacctgaggccgccatccacgccggttgagtcgcgttctgccgcctcccgcctgtggtgcctcctgaactgcgtccgccgtctaggtaagtttaaagctcaggtcgagaccgggcctttgtccggcgctcccttggagcctacctagactcagccggctctccacgctttgcctgaccctgcttgctcaactctacgtctttgtttcgttttctgttctgcgccgttacagatccaagctgtgaccggcgcctac

SEQ ID NO: 42 - DNA, 1494 bp, Homo sapiens
atgcttctcctggtgacaagccttctgctctgtgagttaccacacccagcattcctcctgatcccaggccctgtgcctccctctacagccctcaggtacctcattgaggagctggtcaacatcacccagaaccagaaggctccgctctgcaatggcagcatggtatggagcatcaacctgacagctggcatgtactgtgcagccctggaatccctgatcaacgtgtcaggctgcagtgccatcgagaagacccagaggatgctgagcggattctgcccgcacaaggtctcagctgggcagttttccagcttgcatgtccgagacaccaaaatcgaggtggcccagtttgtaaaggacctgctcttacatttaaagaaactttttcgcgagggacggttcaacgagtccaaatatggtcccccatgcccaccatgcccagcacctgagttcctggggggaccatcagtcttcctgttccccccaaaacccaaggacactctcatgatctcccggacccctgaggtcacgtgcgtggtggtggacgtgagccaggaagaccccgaggtccagttcaactggtacgtggatggcgtggaggtgcataatgccaagacaaagccgcgggaggagcagttcaacagcacgtaccgtgtggtcagcgtcctcaccgtcctgcaccaggactggctgaacggcaaggagtacaagtgcaaggtctccaacaaaggcctcccgtcctccatcgagaaaaccatctccaaagccaaagggcagccccgagagccacaggtgtacaccctgcccccatcccaggaggagatgaccaagaaccaggtcagcctgacctgcctggtcaaaggcttctaccccagcgacatcgccgtggagtgggagagcaatgggcagccggagaacaactacaagaccacgcctcccgtgctggactccgacggctccttcttcctctacagcaggctaaccgtggacaagagcaggtggcaggaggggaatgtcttctcatgctccgtgatgcatgaggctctgcacaaccactacacacagaagagcctctccctgtccctaggtaaaatggccctgattgtgctggggggcgtcgccggcctcctgcttttcattgggctaggcatcttcttcagagtgaagttcagcaggagcgcagacgcccccgcgtaccagcagggccagaaccagctctataacgagctcaatctaggacgaagagaggagtacgatgttttggacaagagacgtggccgggaccctgagatggggggaaagccgagaaggaagaaccctcaggaaggcctgtacaatgaactgcagaaagataagatggcggaggcctacagtgagattgggatgaaaggcgagcgccggaggggcaaggggcacgatggcctttaccagggtctcagtacagccaccaaggacacctacgacgcccttcacatgcaggccctgccccctcgctga

SEQ ID NO: 43 - DNA, 268 bp, Homo sapiens
gacatgataagatacattgatgagtttggacaaaccacaactagaatgcagtgaaaaaaatgctttatttgtgaaatttgtgatgctattgctttatttgtgaaatttgtgatgctattgctttatttgtaaccattataagctgcaataaacaagttaacaacaacaattgcattcattttatgtttcaggttcagggggaggtgtgggaggttttttaaagcaagtaaaacctctacaaatgtggtagatccatttaaatgttagc

SEQ ID NO: 44 - DNA, 748 bp, Homo sapiens
gaagaacatgtgagcaaaaggccagcaaaaggccaggaaccgtaaaaaggccgcgttgctggcgtttttccataggctccgcccccctgacgagcatcacaaaaatcgacgctcaagtcagaggtggcgaaacccgacaggactataaagataccaggcgtttccccctggaagctccctcgtgcgctctcctgttccgaccctgccgcttaccggatacctgtccgcctttctcccttcgggaagcgtggcgctttctcaatgctcacgctgtaggtatctcagttcggtgtaggtcgttcgctccaagctgggctgtgtgcacgaaccccccgttcagcccgaccgctgcgccttatccggtaactatcgtcttgagtccaacccggtaagacacgacttatcgccactggcagcagccactggtaacaggattagcagagcgaggtatgtaggcggtgctacagagttcttgaagtggtggcctaactacggctacactagaagaacagtatttggtatctgcgctctgctgaagccagttaccttcggaaaaagagttggtagctcttgatccggcaaacaaaccaccgctggtagcggtggtttttttgtttgcaagcagcagattacgcgcagaaaaaaaggatctcaagaagatcctttgatcttttctacggggtctgacgctcagtggaacgaaaactcacgttaagggattttggtcatggctagttaattaagctgc

SEQ ID NO: 45 - DNA, 187 bp, Homo sapiens
aataaacaatcattattttcattggatctgtgtgttggttttttgtgtgggcttgggggagggggaggccagaatgactccaagagctacaggaaggcaggtcagagaccccactggacaaacagtggctggactctgcaccataacacacaatcaacaggggagtgagctggatcgagctagagtc

SEQ ID NO: 46 - DNA, 811 bp, Homo sapiens
cgttacataacttacggtaaatggcccgcctggctgaccgcccaacgacccccgcccattgacgtcaataatgacgtatgttcccatagtaacgccaatagggactttccattgacgtcaatgggtggagtatttacggtaaactgcccacttggcagtacatcaagtgtatcatatgccaagtacgccccctattgacgtcaatgacggtaaatggcccgcctggcattatgcccagtacatgaccttatgggactttcctacttggcagtacatctacgtattagtcatcgctattaccatggtgatgcggttttggcagtacatcaatgggcgtggatagcggtttgactcacggggatttccaagtctccaccccattgacgtcaatgggagtttgttttggcaccaaaatcaacgggactttccaaaatgtcgtaacaactccgccccattgacgcaaatgggcggtaggcgtgtacggtgggaggtctatataagcagagctcgtttagtgaaccgtcagatcgcctggagacgccatccacgctgttttgacctccatagaagacaccgggaccgatccagcctccgcggccgggaacggtgcattggaacgcggattccccgtgccaagagtgacgtaagtaccgcctatagagtctataggcccacctagttgtgaccggcgcctagtgttgacaattaatcatcggcatagtataatacgactcactataggagggccaccatgtcgactactaaccttcttctctttcctacagctgagatcaccggtaggagggccatc

SEQ ID NO: 47 - DNA, 2076 bp, Homo sapiens
atgaaaaagcctgaactcaccgcgacgtctgtcgcgaagtttctgatcgaaaagttcgacagcgtctccgacctgatgcagctctcggagggcgaagaatctcgtgctttcagcttcgatgtaggagggcgtggatatgtcctgcgggtaaatagctgcgccgatggtttctacaaagatcgttatgtttatcggcactttgcatcggccgcgctcccgattccggaagtgcttgacattggggaattcagcgagagcctgacctattgcatctcccgccgtgcacagggtgtcacgttgcaagacctgcctgaaaccgaactgcccgctgttctgcaacccgtcgcggagctcatggatgcgatcgctgcggccgatcttagccagacgagcgggttcggcccattcggaccgcaaggaatcggtcaatacactacatggcgtgatttcatatgcgcgattgctgatccccatgtgtatcactggcaaactgtgatggacgacaccgtcagtgcgtccgtcgcgcaggctctcgatgagctgatgctttgggccgaggactgccccgaagtccggcacctcgtgcacgcggatttcggctccaacaatgtcctgacggacaatggccgcataacagcggtcattgactggagcgaggcgatgttcggggattcccaatacgaggtcgccaacatcttcttctggaggccgtggttggcttgtatggagcagcagacgcgctacttcgagcggaggcatccggagcttgcaggatcgccgcggctccgggcgtatatgctccgcattggtcttgaccaactctatcagagcttggttgacggcaatttcgatgatgcagcttgggcgcagggtcgatgcgacgcaatcgtccgatccggagccgggactgtcgggcgtacacaaatcgcccgcagaagcgcggccgtctggaccgatggctgtgtagaagtcgcgtctgcgttcgaccaggctgcgcgttctcgcggccatagcaaccgacgtacggcgttgcgccctcgccggcagcaagaagccacggaagtccgcccggagcagaaaatgcccacgctactgcgggtttatatagacggtccccacgggatggggaaaaccaccaccacgcaactgctggtggccctgggttcgcgcgacgatatcgtctacgtacccgagccgatgacttactggcgggtgctgggggcttccgagacaatcgcgaacatctacaccacacaacaccgcctcgaccagggtgagatatcggccggggacgcggcggtggtaatgacaagcgcccagataacaatgggcatgccttatgccgtgaccgacgccgttctggctcctcatatcgggggggaggctgggagctcacatgccccgcccccggccctcaccctcatcttcgaccgccatcccatcgccgccctcctgtgctacccggccgcgcggtaccttatgggcagcatgaccccccaggccgtgctggcgttcgtggccctcatcccgccgaccttgcccggcaccaacatcgtgcttggggcccttccggaggacagacacatcgaccgcctggccaaacgccagcgccccggcgagcggctggacctggctatgctggctgcgattcgccgcgtttacgggctacttgccaatacggtgcggtatctgcagtgcggcgggtcgtggcgggaggactggggacagctttcggggacggccgtgccgccccagggtgccgagccccagagcaacgcgggcccacgaccccatatcggggacacgttatttaccctgtttcgggcccccgagttgctggcccccaacggcgacctgtataacgtgtttgcctgggccttggacgtcttggccaaacgcctccgttccatgcacgtctttatcctggattacgaccaatcgcccgccggctgccgggacgccctgctgcaacttacctccgggatggtccagacccacgtcaccacccccggctccataccgacgatatgcgacctggcgcgcacgtttgcccgggagatgggggaggctaactga

SEQ ID NO: 48 - DNA, 299 bp, Homo sapiens
gtcgagaattcgctagagggccctattctatagtgtcacctaaatgctagagctcgctgatcagcctcgactgtgccttctagttgccagccatctgttgtttgcccctcccccgtgccttccttgaccctggaaggtgccactcccactgtcctttcctaataaaatgaggaaattgcatcgcattgtctgagtaggtgtcattctattctggggggtggggtggggcaggacagcaagggggaggattgggaagacaatagcaggcatgcgcagggcccaattgctcgagcggccgc

SEQ ID NO: 49 - DNA, 75 bp, Artificial Sequence
  oligonucleotide with homology to foot and mouth disease gene
tctagaggagcatgccagctgttgaattttgaccttcttaagcttgcgggagacgtcgagtccaaccctgggccc

SEQ ID NO: 50 - DNA, 21 bp, Homo sapiens
caagaatcccaaactcaccag

SEQ ID NO: 51 - DNA, 23 bp, Homo sapiens
cgttgatattgctgattaagtcc

SEQ ID NO: 52 - DNA, 24 bp, Homo sapiens
atcccagtaatggttgtcctgcct

SEQ ID NO: 53 - DNA, 24 bp, Homo sapiens
tcttgcttaggttggctgcctagt